European Patent Application EP 4 613 292 A1, published September 10, 2025. Title: Fc 결합성 유닛을 포함하는 화합물 및 이를 이용하여 제조된 컨쥬게이트. Applicant: 앱티스 주식회사. Application WO, filed November 1, 2023. The sequence listing filed with the application follows.

SEQUENCE LISTING (30 sequences)

SEQ ID NO: 1 - protein, 17 aa, synthetic construct
  source 1..17: note = amino acid sequence of Fc binding substance
  SITE 1: note = X is absent or any amino acid residue
  SITE 2: note = X is absent or any amino acid residue
  SITE 3: note = X is any amino acid residue
  SITE 5: note = X is any amino acid residue
  SITE 6: note = X is any amino acid residue
  SITE 8: note = X is a group having structure Xa1
  SITE 10: note = X is glutamic acid residue or asparagine residue
  SITE 13: note = X is tryptophan residue, naphthylalanine residue, or phenylalanine residue
  SITE 15: note = X is any amino acid residue
  SITE 16: note = X is absent or any amino acid residue
  SITE 17: note = X is absent or any amino acid residue
XXXCXXHXGXLVXCXXX

SEQ ID NO: 2 - protein, 15 aa, synthetic construct
  source 1..15: note = amino acid sequence of Fc binding substance
  SITE 1: note = X is L-proline residue
  SITE 4: note = X is any amino acid residue
  SITE 5: note = X is any amino acid residue
  SITE 7: note = X is a group having structure Xa1
  SITE 9: note = X is glutamic acid residue or asparagine residue
  SITE 12: note = X is tryptophan residue, naphthylalanine residue, or phenylalanine residue
  SITE 15: note = X is D-proline residue
XDCXXHXGXLVXCTX

SEQ ID NO: 3 - protein, 15 aa, synthetic construct
  source 1..15: note = amino acid sequence of Fc binding substance
  SITE 4: note = X is any amino acid residue
  SITE 5: note = X is any amino acid residue
  SITE 7: note = X is a group having structure Xa1
  SITE 9: note = X is glutamic acid residue or asparagine residue
  SITE 12: note = X is tryptophan residue, naphthylalanine residue, or phenylalanine residue
CDCXXHXGXLVXCTC

SEQ ID NO: 4 - protein, 13 aa, synthetic construct
  source 1..13: note = amino acid sequence of Fc binding substance
  SITE 3: note = X is any amino acid residue
  SITE 4: note = X is any amino acid residue
  SITE 6: note = X is a group having structure Xa1
  SITE 8: note = X is glutamic acid residue or asparagine residue
  SITE 11: note = X is tryptophan residue, naphthylalanine residue, or phenylalanine residue
DCXXHXGXLVXCT

SEQ ID NO: 5 - protein, 13 aa, synthetic construct
  source 1..13: note = amino acid sequence of Fc binding substance
  SITE 6: note = X is a group having structure Xa1
DCAWHXGELVWCT

SEQ ID NO: 6 - protein, 13 aa, synthetic construct
  source 1..13: note = amino acid sequence of Fc binding substance
  SITE 6: note = X is diaminopropionic acid
DCAWHXGELVWCT

SEQ ID NO: 7 - protein, 13 aa, synthetic construct
  source 1..13: note = amino acid sequence of Fc binding substance
  SITE 6: note = X is diaminobytyric acid
DCAWHXGELVWCT

SEQ ID NO: 8 - protein, 13 aa, synthetic construct
  source 1..13: note = amino acid sequence of Fc binding substance
  SITE 6: note = X is ornithine residue
DCAWHXGELVWCT

SEQ ID NO: 9 - protein, 13 aa, synthetic construct
  source 1..13: note = amino acid sequence of Fc binding substance
DCAWHKGELVWCT

SEQ ID NO: 10 - protein, 7 aa, synthetic construct
  source 1..7: note = amino acid sequence in IgG Fc region
KPKDTLM

SEQ ID NO: 11 - protein, 8 aa, synthetic construct
  source 1..8: note = amino acid sequence in IgG Fc region
MHEALHNH

SEQ ID NO: 12 - protein, 9 aa, synthetic construct
  source 1..9: note = amino acid sequence in IgG Fc region
MHEALHNHY

SEQ ID NO: 13 - protein, 16 aa, synthetic construct
  source 1..16: note = amino acid sequence in IgG Fc region
GPSVFLFPPKPKDTLM

SEQ ID NO: 14 - protein, 208 aa, synthetic construct
  source 1..208: note = amino acid sequence in CH2-CH3 domain of human IgG1 Fc region
GPSVFLFPPKPKDTLMISRTPEVTCVVVDVSHEDPEVKFNWYVDGVEVHNAKTKPREEQYNSTYRVVSVLTVLHQDWLNGKEYKCKVSNKALPAPIEKTISKAKGQPREPQVYTLPPSREEMTKNQVSLTCLVKGFYPSDIAVEWESNGQPENNYKTTPPVLDSDGSFFLYSKLTVDKSRWQQGNVFSCSVMHEALHNHYTQKSLSLS

SEQ ID NO: 15 - protein, 208 aa, synthetic construct
  source 1..208: note = amino acid sequence in CH2-CH3 domain of human IgG2 Fc region
GPSVFLFPPKPKDTLMISRTPEVTCVVVDVSHEDPEVQFNWYVDGVEVHNAKTKPREEQFNSTFRVVSVLTVVHQDWLNGKEYKCKVSNKGLPAPIEKTISKTKGQPREPQVYTLPPSREEMTKNQVSLTCLVKGFYPSDIAVEWESNGQPENNYKTTPPMLDSDGSFFLYSKLTVDKSRWQQGNVFSCSVMHEALHNHYTQKSLSLS

SEQ ID NO: 16 - protein, 208 aa, synthetic construct
  source 1..208: note = amino acid sequence in CH2-CH3 domain of human IgG3 Fc region
GPSVFLFPPKPKDTLMISRTPEVTCVVVDVSHEDPEVQFKWYVDGVEVHNAKTKPREEQYNSTFRVVSVLTVLHQDWLNGKEYKCKVSNKALPAPIEKTISKTKGQPREPQVYTLPPSREEMTKNQVSLTCLVKGFYPSDIAVEWESSGQPENNYNTTPPMLDSDGSFFLYSKLTVDKSRWQQGNIFSCSVMHEALHNHFTQKSLSLS

SEQ ID NO: 17 - protein, 208 aa, synthetic construct
  source 1..208: note = amino acid sequence in CH2-CH3 domain of human IgG4 Fc region
GPSVFLFPPKPKDTLMISRTPEVTCVVVDVSQEDPEVQFNWYVDGVEVHNAKTKPREEQFNSTYRVVSVLTVLHQDWLNGKEYKCKVSNKGLPSSIEKTISKAKGQPREPQVYTLPPSQEEMTKNQVSLTCLVKGFYPSDIAVEWESNGQPENNYKTTPPVLDSDGSFFLYSRLTVDKSRWQEGNVFSCSVMHEALHNHYTQKSLSLS

SEQ ID NO: 18 - protein, 208 aa, synthetic construct
  source 1..208: note = amino acid sequence in CH2-CH3 domain of Herceptin Fc region
GPSVFLFPPKPKDTLMISRTPEVTCVVVDVSHEDPEVKFNWYVDGVEVHNAKTKPREEQYNSTYRVVSVLTVLHQDWLNGKEYKCKVSNKALPAPIEKTISKAKGQPREPQVYTLPPSRDELTKNQVSLTCLVKGFYPSDIAVEWESNGQPENNYKTTPPVLDSDGSFFLYSKLTVDKSRWQQGNVFSCSVMHEALHNHYTQKSLSLS

SEQ ID NO: 19 - protein, 5 aa, synthetic construct
  source 1..5: note = CDRH1 of anti-CLDN18.2 antibody
TYGVH

SEQ ID NO: 20 - protein, 16 aa, synthetic construct
  source 1..16: note = CDRH2 of anti-CLDN18.2 antibody
VIWAGGSTNYNSALMS

SEQ ID NO: 21 - protein, 10 aa, synthetic construct
  source 1..10: note = CDRH3 of anti-CLDN18.2 antibody
AAYYGNGLDY

SEQ ID NO: 22 - protein, 17 aa, synthetic construct
  source 1..17: note = CDRL1 of anti-CLDN18.2 antibody
KSSQTLLNSGNQKNYLT

SEQ ID NO: 23 - protein, 7 aa, synthetic construct
  source 1..7: note = CDRL2 of anti-CLDN18.2 antibody
WASTGES

SEQ ID NO: 24 - protein, 9 aa, synthetic construct
  source 1..9: note = CDRL3 of anti-CLDN18.2 antibody
QNAYFYPFT

SEQ ID NO: 25 - protein, 448 aa, synthetic construct
  source 1..448: note = anti-CLDN 18.2 antibody Heavy chain
QVQLVESGGGVVQPGRSLRLSCAASGFSLTTYGVHWVRQAPGKGLEWVAVIWAGGSTNYNSALMSRFTISRDNSKNTLYLQMNSLRAEDTAVYYCARAAYYGNGLDYWGQGTMVTVSSASTKGPSVFPLAPSSKSTSGGTAALGCLVKDYFPEPVTVSWNSGALTSGVHTFPAVLQSSGLYSLSSVVTVPSSSLGTQTYICNVNHKPSNTKVDKRVEPKSCDKTHTCPPCPAPELLGGPSVFLFPPKPKDTLMISRTPEVTCVVVDVSHEDPEVKFNWYVDGVEVHNAKTKPREEQYNSTYRVVSVLTVLHQDWLNGKEYKCKVSNKALPAPIEKTISKAKGQPREPQVYTLPPSRDELTKNQVSLTCLVKGFYPSDIAVEWESNGQPENNYKTTPPVLDSDGSFFLYSKLTVDKSRWQQGNVFSCSVMHEALHNHYTQKSLSLSPGK

SEQ ID NO: 26 - protein, 220 aa, synthetic construct
  source 1..220: note = anti-CLDN 18.2 antibody Light chain
DIVMTQSPLSLPVTPGEPASISCKSSQTLLNSGNQKNYLTWYLQKPGQSPQLLIYWASTGESGVPDRFSGSGSGTDFTLKISRVEAEDVGVYYCQNAYFYPFTFGGGTKVEIKRTVAAPSVFIFPPSDEQLKSGTASVVCLLNNFYPREAKVQWKVDNALQSGNSQESVTEQDSKDSTYSLSSTLTLSKADYEKHKVYACEVTHQGLSSPVTKSFNRGEC

SEQ ID NO: 27 - protein, 5 aa, synthetic construct
  source 1..5: note = Target region
PKPKD

SEQ ID NO: 28 - skipped

SEQ ID NO: 29 - DNA, 783 bp, synthetic construct
  source 1..783: mol_type = other DNA; note = nucleic acid sequence encoding CLDN 18.1
atgtccaccaccacatgccaagtggtggcgttcctcctgtccatcctggggctggccggctgcatcgcggccaccgggatggacatgtggagcacccaggacctgtacgacaaccccgtcacctccgtgttccagtacgaagggctctggaggagctgcgtgaggcagagttcaggcttcaccgaatgcaggccctatttcaccatcctgggacttccagccatgctgcaggcagtgcgagccctgatgatcgtaggcatcgtcctgggtgccattggcctcctggtatccatctttgccctgaaatgcatccgcattggcagcatggaggactctgccaaagccaacatgacactgacctccgggatcatgttcattgtctcaggtctttgtgcaattgctggagtgtctgtgtttgccaacatgctggtgactaacttctggatgtccacagctaacatgtacaccggcatgggtgggatggtgcagactgttcagaccaggtacacatttggtgcggctctgttcgtgggctgggtcgctggaggcctcacactaattgggggtgtgatgatgtgcatcgcctgccggggcctggcaccagaagaaaccaactacaaagccgtttcttatcatgcctcaggccacagtgttgcctacaagcctggaggcttcaaggccagcactggctttgggtccaacaccaaaaacaagaagatatacgatggaggtgcccgcacagaggacgaggtacaatcttatccttccaagcacgactatgtg

SEQ ID NO: 30 - DNA, 786 bp, synthetic construct
  source 1..786: mol_type = other DNA; note = nucleic acid sequence encoding CLDN 18.2
atggccgtgactgcctgtcagggcttggggttcgtggtttcactgattgggattgcgggcatcattgctgccacctgcatggaccagtggagcacccaagacttgtacaacaaccccgtaacagctgttttcaactaccaggggctgtggcgctcctgtgtccgagagagctctggcttcaccgagtgccggggctacttcaccctgctggggctgccagccatgctgcaggcagtgcgagccctgatgatcgtaggcatcgtcctgggtgccattggcctcctggtatccatctttgccctgaaatgcatccgcattggcagcatggaggactctgccaaagccaacatgacactgacctccgggatcatgttcattgtctcaggtctttgtgcaattgctggagtgtctgtgtttgccaacatgctggtgactaacttctggatgtccacagctaacatgtacaccggcatgggtgggatggtgcagactgttcagaccaggtacacatttggtgcggctctgttcgtgggctgggtcgctggaggcctcacactaattgggggtgtgatgatgtgcatcgcctgccggggcctggcaccagaagaaaccaactacaaagccgtttcttatcatgcctcaggccacagtgttgcctacaagcctggaggcttcaaggccagcactggctttgggtccaacaccaaaaacaagaagatatacgatggaggtgcccgcacagaggacgaggtacaatcttatccttccaagcacgactatgtgtaa